European Patent Application EP 4 534 664 A1, published April 9, 2025. Title: Novel variant of phosphoenolpyruvate caboxylase and method for producing 5'-inosinic acid using the same. Applicant: DAESANG CORPORATION. The sequence listing filed with the application follows.

SEQUENCE LISTING (7 sequences)

SEQ ID NO: 1 - DNA, 2805 bp, synthetic construct
  source 1..2805: mol_type = other DNA
atgttcaatagcactgacgtttcgctggaaaggaaccccactgcaatgagtgaacaggtgcgcgatgatatccgactgctaggacgcatcctcggccgagtaattgccgagcaagaaggcgaagatgtatttgagttggtggaaagcactcgccgcttggccttcggggtggcgcgcggtgaggaaaaagctgaggctttgctggcgaccttccggactatcgatgaaaaccgcatcaacctcgttgcgcgttctttcagccactttgcgctgatggcgaatatcgcagaggacctcgacgatgaaacggcgcttgcagcccgcgaggatgctggtgcacaggctcccgatgcttccctgcacggagttttgggcaagctcaaggcggcgaaagacatcaaaacaagtgatgtcacccgtatcttggatgccgcgcaagtctcccctgtttttaccgcacaccccacggagacacggcgtcgtacggtatttgatgtccaggagcgcatcgtggcgctattgcgtgagcgccacagcatcttggcccaaccgcaaacagcaaggcttgaagcccgtcttgctgagattgaacgcgaggctcacctgcgcatgaccatcctgtggcaaaccgcgttaattcgcattgcacggccacagatcgaagatgaagtaaacgtaggtctgcgctacttcaagcgcagcctcttagagcaggtaccggcgattaaccgcgacaccatcgccgggcttcgcgatgtcttcggcgcatcagtgcccaaccggcaagttgtgcgcacagggtcatggatcggcggcgaccacgatggcaatccttatgtcaccggcgatactttgacctacgcgacgcgacaggccgcggataccatcctggaatactacgttgatgagctcgcagcactagaaaaggaactgagcttatcagaccgctattcagaaagttccgcggaattacaagaactggccacgcgcgggagaaacgatattccaagtcgcgtcgatgagccttaccgcagggcaatccacggagtgcacggacgcatgatagctacccgcgcagccgttgcaggagaagccgcagctgagtctggggaattttcaccttatgcctccccgacccagtttcgcacggatttgcaggttattgaccggtctttgcggcaatttaatgatgcgatcatcgccgacgataggctgctgcgaattctttctgccgtggatacttttggcttccacctcaatgctttggatctgcgtcagaactcggagtctttcgaggccgtcttggacgaacttttcgctgccgcgggcgttactgcaccagatgccggatacgccagcctggatgagagcgccaagcgtgaactactagtagctgagctcacctctgctcgctcactggtcttcccgtggtctcaagacttcagtgcagacacggaacgcgaactagggatcttccgggcagcagcccaggccgtcgagttactggggccaggtgttgtcccacactgcattgtttcaatgaccggtacagtcagcgatattttggaaccgatggtactgctcaaagaagtaggcatcataagctttaacccagcccagcaacgcctcgttggttcagtggacatcgcaccgctttttgaaaccattgaagacttaaaggctggcgcggagatccttcaagaactatgggaagttgacctttaccgcggatacttgcgcgggcgcgaagacgtccaagaagtcgtgttggggtattccgactccaataaagacggcgggtatttgtctgcgaattgggctttatatgatgcgcagctagccatcgtcaaggcctgcgatacgcacggcatcgggttgcgcttttcacatggccgcggcggtgctgtgggtcgcggtggcgggccgacgtacgatgccatcttggcccagcccgaaggtgcggtccggggcagcgtgcgtattaccgagcaaggtgaggtcatctctgcccgctacgacacagcgagtaccgcgcgccgccacctggaagcttttgtcgcgggcacgctagaagcctctctactggatactgaaaagctaaaagagcctgaacgcgcctatggcatcatgcgggatatcgcctcgctggccggtgagaaatatgcgcaattggtgcgcgatgactccgggtttatcgactacttcacgcaatccacgccattgcacgaaattggcgacctcaatatgggatcacgtccaactgctcgcaagcagaccgaatccatcggtgacttgcgcgcgattccatgggtcctgtcatggtcgcagtcgcgcgttaacctgccgggctggttcggagtgggcacaggcatcatgcgctgggctggcgaagacgagacccgctggcaagatttgcgcaagctttatcaggcatggccgttctttcgttccgtgctcgacaacatggcgcaggtcatggggaaagcgtcgatgaatctcgcaaagatctactccacgcttgtcgatgaccccacggtctcccagcgcgtgtttaacaccatcctggacgaatacgaattaaccaaagaagtattcttccgcatcactggtcatgattcgctcatggctggtaatgagcgtttggagcgttcagtacagcgacgctatccatacttactgccgctcaacgccatccagattgagttgctgcgccgctaccgtgcgggcgaggatacattcttggtctctaagaccatccaggtgaccatgaacggacttgcgacaggactacgcacctcaggctag

SEQ ID NO: 2 - protein, 934 aa, synthetic construct
MFNSTDVSLERNPTAMSEQVRDDIRLLGRILGRVIAEQEGEDVFELVESTRRLAFGVARGEEKAEALLATFRTIDENRINLVARSFSHFALMANIAEDLDDETALAAREDAGAQAPDASLHGVLGKLKAAKDIKTSDVTRILDAAQVSPVFTAHPTETRRRTVFDVQERIVALLRERHSILAQPQTARLEARLAEIEREAHLRMTILWQTALIRIARPQIEDEVNVGLRYFKRSLLEQVPAINRDTIAGLRDVFGASVPNRQVVRTGSWIGGDHDGNPYVTGDTLTYATRQAADTILEYYVDELAALEKELSLSDRYSESSAELQELATRGRNDIPSRVDEPYRRAIHGVHGRMIATRAAVAGEAAAESGEFSPYASPTQFRTDLQVIDRSLRQFNDAIIADDRLLRILSAVDTFGFHLNALDLRQNSESFEAVLDELFAAAGVTAPDAGYASLDESAKRELLVAELTSARSLVFPWSQDFSADTERELGIFRAAAQAVELLGPGVVPHCIVSMTGTVSDILEPMVLLKEVGIISFNPAQQRLVGSVDIAPLFETIEDLKAGAEILQELWEVDLYRGYLRGREDVQEVVLGYSDSNKDGGYLSANWALYDAQLAIVKACDTHGIGLRFSHGRGGAVGRGGGPTYDAILAQPEGAVRGSVRITEQGEVISARYDTASTARRHLEAFVAGTLEASLLDTEKLKEPERAYGIMRDIASLAGEKYAQLVRDDSGFIDYFTQSTPLHEIGDLNMGSRPTARKQTESIGDLRAIPWVLSWSQSRVNLPGWFGVGTGIMRWAGEDETRWQDLRKLYQAWPFFRSVLDNMAQVMGKASMNLAKIYSTLVDDPTVSQRVFNTILDEYELTKEVFFRITGHDSLMAGNERLERSVQRRYPYLLPLNAIQIELLRRYRAGEDTFLVSKTIQVTMNGLATGLRTSG

SEQ ID NO: 3 - DNA, 2805 bp, Corynebacterium stationis
  source 1..2805: mol_type = genomic DNA
atgttcaatagcactgacgtttcgctggaaaggaaccccactgcaatgagtgaacaggtgcgcgatgatatccgactgctaggacgcatcctcggccgagtaattgccgagcaagaaggcgaagatgtatttgagttggtggaaagcactcgccgcttggccttcggggtggcgcgcggtgaggaaaaagctgaggctttgctggcgaccttccggactatcgatgaaaaccgcatcaacctcgttgcgcgttctttcagccactttgcgctgatggcgaatatcgcagaggacctcgacgatgaaacggcgcttgcagcccgcgaggatgctggtgcacaggctcccgatgcttccctgcacggagttttgggcaagctcaaggcggcgaaagacatcaaaacaagtgatgtcacccgtatcttggatgccgcgcaagtctcccctgtttttaccgcacaccccacggagacacggcgtcgtacggtatttgatgtccaggagcgcatcgtggcgctattgcgtgagcgccacagcatcttggcccaaccgcaaacagcaaggcttgaagcccgtcttgctgagattgaacgcgaggctcacctgcgcatgaccatcctgtggcaaaccgcgttaattcgcattgcacggccacagatcgaagatgaagtaaacgtaggtctgcgctacttcaagcgcagcctcttagagcaggtaccggcgattaaccgcgacaccatcgccgggcttcgcgatgtcttcggcgcatcagtgcccaaccggcaagttgtgcgcacagggtcatggatcggcggcgaccacgatggcaatccttatgtcaccggcgatactttgacctacgcgacgcgacaggccgcggataccatcctggaatactacgttgatgagctcgcagcactagaaaaggaactgagcttatcagaccgctattcagaaagttccgcggaattacaagaactggccacgcgcgggagaaacgatattccaagtcgcgtcgatgagccttaccgcagggcaatccacggagtgcacggacgcatgatagctacccgcgcagccgttgcaggagaagccgcagctgagtctggggaattttcaccttatgcctccccgacccagtttcgcacggatttgcaggttattgaccggtctttgcggcaatttaatgatgcgatcatcgccgacgataggctgctgcgaattctttctgccgtggatacttttggcttccacctcaatgctttggatctgcgtcagaactcggagtctttcgaggccgtcttggacgaacttttcgctgccgcgggcgttactgcaccagatgccggatacgccagcctggatgagagcgccaagcgtgaactactagtagctgagctcacctctgctcgcccactggtcttcccgtggtctcaagacttcagtgcagacacggaacgcgaactagggatcttccgggcagcagcccaggccgtcgagttactggggccaggtgttgtcccacactgcattgtttcaatgaccggtacagtcagcgatattttggaaccgatggtactgctcaaagaagtaggcatcataagctttaacccagcccagcaacgcctcgttggttcagtggacatcgcaccgctttttgaaaccattgaagacttaaaggctggcgcggagatccttcaagaactatgggaagttgacctttaccgcggatacttgcgcgggcgcgaagacgtccaagaagtcgtgttggggtattccgactccaataaagacggcgggtatttgtctgcgaattgggctttatatgatgcgcagctagccatcgtcaaggcctgcgatacgcacggcatcgggttgcgcttttcacatggccgcggcggtgctgtgggtcgcggtggcgggccgacgtacgatgccatcttggcccagcccgaaggtgcggtccggggcagcgtgcgtattaccgagcaaggtgaggtcatctctgcccgctacggcacagcgagtaccgcgcgccgccacctggaagcttttgtcgcgggcacgctagaagcctctctactggatactgaaaagctaaaagagcctgaacgcgcctatggcatcatgcgggatatcgcctcgctggccggtgagaaatatgcgcaattggtgcgcgatgactccgggtttatcgactacttcacgcaatccacgccattgcacgaaattggcgacctcaatatgggatcacgtccaactgctcgcaagcagaccgaatccatcggtgacttgcgcgcgattccatgggtcctgtcatggtcgcagtcgcgcgttaacctgccgggctggttcggagtgggcacaggcatcatgcgctgggctggcgaagacgagacccgctggcaagatttgcgcaagctttatcaggcatggccgttctttcgttccgtgctcgacaacatggcgcaggtcatggggaaagcgtcgatgaatctcgcaaagatctactccacgcttgtcgatgaccccacggtctcccagcgcgtgtttaacaccatcctggacgaatacgaattaaccaaagaagtattcttccgcatcactggtcatgattcgctcatggctggtaatgagcgtttggagcgttcagtacagcgacgctatccatacttactgccgctcaacgccatccagattgagttgctgcgccgctaccgtgcgggcgaggatacattcttggtctctaagaccatccaggtgaccatgaacggacttgcgacaggactacgcacctcaggctag

SEQ ID NO: 4 - protein, 934 aa, Corynebacterium stationis
MFNSTDVSLERNPTAMSEQVRDDIRLLGRILGRVIAEQEGEDVFELVESTRRLAFGVARGEEKAEALLATFRTIDENRINLVARSFSHFALMANIAEDLDDETALAAREDAGAQAPDASLHGVLGKLKAAKDIKTSDVTRILDAAQVSPVFTAHPTETRRRTVFDVQERIVALLRERHSILAQPQTARLEARLAEIEREAHLRMTILWQTALIRIARPQIEDEVNVGLRYFKRSLLEQVPAINRDTIAGLRDVFGASVPNRQVVRTGSWIGGDHDGNPYVTGDTLTYATRQAADTILEYYVDELAALEKELSLSDRYSESSAELQELATRGRNDIPSRVDEPYRRAIHGVHGRMIATRAAVAGEAAAESGEFSPYASPTQFRTDLQVIDRSLRQFNDAIIADDRLLRILSAVDTFGFHLNALDLRQNSESFEAVLDELFAAAGVTAPDAGYASLDESAKRELLVAELTSARPLVFPWSQDFSADTERELGIFRAAAQAVELLGPGVVPHCIVSMTGTVSDILEPMVLLKEVGIISFNPAQQRLVGSVDIAPLFETIEDLKAGAEILQELWEVDLYRGYLRGREDVQEVVLGYSDSNKDGGYLSANWALYDAQLAIVKACDTHGIGLRFSHGRGGAVGRGGGPTYDAILAQPEGAVRGSVRITEQGEVISARYGTASTARRHLEAFVAGTLEASLLDTEKLKEPERAYGIMRDIASLAGEKYAQLVRDDSGFIDYFTQSTPLHEIGDLNMGSRPTARKQTESIGDLRAIPWVLSWSQSRVNLPGWFGVGTGIMRWAGEDETRWQDLRKLYQAWPFFRSVLDNMAQVMGKASMNLAKIYSTLVDDPTVSQRVFNTILDEYELTKEVFFRITGHDSLMAGNERLERSVQRRYPYLLPLNAIQIELLRRYRAGEDTFLVSKTIQVTMNGLATGLRTSG

SEQ ID NO: 5 - DNA, 5719 bp, synthetic construct
  source 1..5719: mol_type = other DNA
tgccgcaagcactcagggcgcaagggctgctaaaggaagcggaacacgtagaaagccagtccgcagaaacggtgctgaccccggatgaatgtcagctactgggctatctggacaagggaaaacgcaagcgcaaagagaaagcaggtagcttgcagtgggcttacatggcgatagctagactgggcggttttatggacagcaagcgaaccggaattgccagctggggcgccctctggtaaggttgggaagccctgcaaagtaaactggatggctttcttgccgccaaggatctgatggcgcaggggatcaagatctgatcaagagacaggatgaggatcgtttcgcatgattgaacaagatggattgcacgcaggttctccggccgcttgggtggagaggctattcggctatgactgggcacaacagacaatcggctgctctgatgccgccgtgttccggctgtcagcgcaggggcgcccggttctttttgtcaagaccgacctgtccggtgccctgaatgaactccaagacgaggcagcgcggctatcgtggctggccacgacgggcgttccttgcgcagctgtgctcgacgttgtcactgaagcgggaagggactggctgctattgggcgaagtgccggggcaggatctcctgtcatctcaccttgctcctgccgagaaagtatccatcatggctgatgcaatgcggcggctgcatacgcttgatccggctacctgcccattcgaccaccaagcgaaacatcgcatcgagcgagcacgtactcggatggaagccggtcttgtcgatcaggatgatctggacgaagagcatcaggggctcgcgccagccgaactgttcgccaggctcaaggcgcggatgcccgacggcgaggatctcgtcgtgacccatggcgatgcctgcttgccgaatatcatggtggaaaatggccgcttttctggattcatcgactgtggccggctgggtgtggcggaccgctatcaggacatagcgttggctacccgtgatattgctgaagagcttggcggcgaatgggctgaccgcttcctcgtgctttacggtatcgccgctcccgattcgcagcgcatcgccttctatcgccttcttgacgagttcttctgagcgggactctggggttcgctagaggatcgatcctttttaacccatcacatatacctgccgttcactattatttagtgaaatgagatattatgatattttctgaattgtgattaaaaaggcaactttatgcccatgcaacagaaactataaaaaatacagagaatgaaaagaaacagatagattttttagttctttaggcccgtagtctgcaaatccttttatgattttctatcaaacaaaagaggaaaatagaccagttgcaatccaaacgagagtctaatagaatgaggtcgaaaagtaaatcgcgcgggtttgttactgataaagcaggcaagacctaaaatgtgtaaagggcaaagtgtatactttggcgtcaccccttacatattttaggtctttttttattgtgcgtaactaacttgccatcttcaaacaggagggctggaagaagcagaccgctaacacagtacataaaaaaggagacatgaacgatgaacatcaaaaagtttgcaaaacaagcaacagtattaacctttactaccgcactgctggcaggaggcgcaactcaagcgtttgcgaaagaaacgaaccaaaagccatataaggaaacatacggcatttcccatattacacgccatgatatgctgcaaatccctgaacagcaaaaaaatgaaaaatatcaagtttctgaatttgattcgtccacaattaaaaatatctcttctgcaaaaggcctggacgtttgggacagctggccattacaaaacgctgacggcactgtcgcaaactatcacggctaccacatcgtctttgcattagccggagatcctaaaaatgcggatgacacatcgatttacatgttctatcaaaaagtcggcgaaacttctattgacagctggaaaaacgctggccgcgtctttaaagacagcgacaaattcgatgcaaatgattctatcctaaaagaccaaacacaagaatggtcaggttcagccacatttacatctgacggaaaaatccgtttattctacactgatttctccggtaaacattacggcaaacaaacactgacaactgcacaagttaacgtatcagcatcagacagctctttgaacatcaacggtgtagaggattataaatcaatctttgacggtgacggaaaaacgtatcaaaatgtacagcagttcatcgatgaaggcaactacagctcaggcgacaaccatacgctgagagatcctcactacgtagaagataaaggccacaaatacttagtatttgaagcaaacactggaactgaagatggctaccaaggcgaagaatctttatttaacaaagcatactatggcaaaagcacatcattcttccgtcaagaaagtcaaaaacttctgcaaagcgataaaaaacgcacggctgagttagcaaacggcgctctcggtatgattgagctaaacgatgattacacactgaaaaaagtgatgaaaccgctgattgcatctaacacagtaacagatgaaattgaacgcgcgaacgtctttaaaatgaacggcaaatggtacctgttcactgactcccgcggatcaaaaatgacgattgacggcattacgtctaacgatatttacatgcttggttatgtttctaattctttaactggcccatacaagccgctgaacaaaactggccttgtgttaaaaatggatcttgatcctaacgatgtaacctttacttactcacacttcgctgtacctcaagcgaaaggaaacaatgtcgtgattacaagctatatgacaaacagaggattctacgcagacaaacaatcaacgtttgcgccgagcttcctgctgaacatcaaaggcaagaaaacatctgttgtcaaagacagcatccttgaacaaggacaattaacagttaacaaataaaaacgcaaaagaaaatgccgatgggtaccgagcgaaatgaccgaccaagcgacgcccaacctgccatcacgagatttcgattccaccgccgccttctatgaaaggttgggcttcggaatcgttttccgggacgccctcgcggacgtgctcatagtccacgacgcccgtgattttgtagccctggccgacggccagcaggtaggccgacaggctcatgccggccgccgccgccttttcctcaatcgctcttcgttcgtctggaaggcagtacaccttgataggtgggctgcccttcctggttggcttggtttcatcagccatccgcttgccctcatctgttacgccggcggtagccggccagcctcgcagagcaggattcccgttgagcaccgccaggtgcgaataagggacagtgaagaaggaacacccgctcgcgggtgggcctacttcacctatcctgcccggctgacgccgttggatacaccaaggaaagtctacacgaaccctttggcaaaatcctgtatatcgtgcgaaaaaggatggatataccgaaaaaatcgctataatgaccccgaagcagggttatgcagcggaaaagcgctgcttccctgctgttttgtggaatatctaccgactggaaacaggcaaatgcaggaaattactgaactgaggggacaggcgagagacgatgccaaagagctcctgaaaatctcgataactcaaaaaatacgcccggtagtgatcttatttcattatggtgaaagttggaacctcttacgtgccgatcaacgtctcattttcgccaaaagttggcccagggcttcccggtatcaacagggacaccaggatttatttattctgcgaagtgatcttccgtcacaggtatttattcggcgcaaagtgcgtcgggtgatgctgccaacttactgatttagtgtatgatggtgtttttgaggtgctccagtggcttctgtttctatcagctcctgaaaatctcgataactcaaaaaatacgcccggtagtgatcttatttcattatggtgaaagttggaacctcttacgtgccgatcaacgtctcattttcgccaaaagttggcccagggcttcccggtatcaacagggacaccaggatttatttattctgcgaagtgatcttccgtcacaggtatttattcggcgcaaagtgcgtcgggtgatgctgccaacttactgatttagtgtatgatggtgtttttgaggtgctccagtggcttctgtttctatcagggctggatgatcctccagcgcggggatctcatgctggagttcttcgcccaccccaaaaggatctaggtgaagatcctttttgataatctcatgaccaaaatcccttaacgtgagttttcgttccactgagcgtcagaccccgtagaaaagatcaaaggatcttcttgagatcctttttttctgcgcgtaatctgctgcttgcaaacaaaaaaaccaccgctaccagcggtggtttgtttgccggatcaagagctaccaactctttttccgaaggtaactggcttcagcagagcgcagataccaaatactgttcttctagtgtagccgtagttaggccaccacttcaagaactctgtagcaccgcctacatacctcgctctgctaatcctgttaccagtggctgctgccagtggcgataagtcgtgtcttaccgggttggactcaagacgatagttaccggataaggcgcagcggtcgggctgaacggggggttcgtgcacacagcccagcttggagcgaacgacctacaccgaactgagatacctacagcgtgagctatgagaaagcgccacgcttcccgaagggagaaaggcggacaggtatccggtaagcggcagggtcggaacaggagagcgcacgagggagcttccagggggaaacgcctggtatctttatagtcctgtcgggtttcgccacctctgacttgagcgtcgatttttgtgatgctcgtcaggggggcggagcctatggaaaaacgccagcaacgcggcctttttacggttcctggccttttgctggccttttgctcacatgttctttcctgcgttatcccctgattctgtggataaccgtattaccgcctttgagtgagctgataccgctcgccgcagccgaacgaccgagcgcagcgagtcagtgagcgaggaagcggaagagcgcccaatacgcaaaccgcctctccccgcgcgttggccgattcattaatgcagctggcacgacaggtttcccgactggaaagcgggcagtgagcgcaacgcaattaatgtgagttagctcactcattaggcaccccaggctttacactttatgcttccggctcgtatgttgtgtggaattgtgagcggataacaatttcacacaggaaacagctatgacatgattacgccaagcttgcatgcctgcaggtcgactctagaggatccccgggtaccgagctcgaattcactggccgtcgttttacaacgtcgtgactgggaaaaccctggcgttacccaacttaatcgccttgcagcacatccccctttcgccagctggcgtaatagcgaagaggcccgcaccgatcgcccttcccaacagttgcgcagcctgaatggcgaatggcgataagctagcttcacgc

SEQ ID NO: 6 - DNA, 20 bp, synthetic construct
  source 1..20: mol_type = other DNA
ctctgctcgctcactggtct

SEQ ID NO: 7 - DNA, 21 bp, synthetic construct
  source 1..21: mol_type = other DNA
tactcgctgtgtcgtagcggg